European Patent Application EP 4 357 780 A1, published April 24, 2024. Title: Immunoassay method and immunoassay kit for SARS-CoV-2. Applicant: Sekisui Medical Co., Ltd. The sequence listing filed with the application follows.

SEQUENCE LISTING (85 sequences)

SEQ ID NO: 1 - protein, 18 aa, Unknown
  SARS-CoV-2
KQQTVTLLPAADLDDFSK

SEQ ID NO: 2 - protein, 12 aa, Unknown
  SARS-CoV-2
AADLDDFSKQLQ

SEQ ID NO: 3 - protein, 10 aa, Unknown
  S32213HCCDR1
GFSLSTSGMG

SEQ ID NO: 4 - protein, 7 aa, Unknown
  S32213HCCDR2
IYWDDDK

SEQ ID NO: 5 - protein, 11 aa, Unknown
  S32213HCCDR3
ARRDYGYNFDY

SEQ ID NO: 6 - protein, 7 aa, Unknown
  S32213LCCDR1
SSVSSTY

SEQ ID NO: 7 - protein, 3 aa, Unknown
  S32213LCCDR2
STS

SEQ ID NO: 8 - protein, 9 aa, Unknown
  S32213LCCDR3
HQWSSYPPT

SEQ ID NO: 9 - protein, 8 aa, Unknown
  S32217HCCDR1
GFTFSDYY

SEQ ID NO: 10 - protein, 8 aa, Unknown
  S32217HCCDR2
ITDGDNYT

SEQ ID NO: 11 - protein, 14 aa, Unknown
  S32217HCCDR3
ARDGNYYASSPFTY

SEQ ID NO: 12 - protein, 9 aa, Unknown
  S32217LCCDR1
TGAVTTSNY

SEQ ID NO: 13 - protein, 3 aa, Unknown
  S32217LCCDR2
GTN

SEQ ID NO: 14 - protein, 9 aa, Unknown
  S32217LCCDR3
ALWYSNHWV

SEQ ID NO: 15 - protein, 8 aa, Unknown
  S32223HCCDR1
GFTFSDYY

SEQ ID NO: 16 - protein, 8 aa, Unknown
  S32223HCCDR2
ISDGYSYT

SEQ ID NO: 17 - protein, 13 aa, Unknown
  S32223HCCDR3
ARDQDYFGSSLAY

SEQ ID NO: 18 - protein, 9 aa, Unknown
  S32223LCCDR1
TGAVTTSNY

SEQ ID NO: 19 - protein, 3 aa, Unknown
  S32223LCCDR2
GTN

SEQ ID NO: 20 - protein, 9 aa, Unknown
  S32223LCCDR3
ALWYSNRWV

SEQ ID NO: 21 - protein, 419 aa, Unknown
  SARS-CoV-2
MSDNGPQNQRNAPRITFGGPSDSTGSNQNGERSGARSKQRRPQGLPNNTASWFTALTQHGKEDLKFPRGQGVPINTNSSPDDQIGYYRRATRRIRGGDGKMKDLSPRWYFYYLGTGPEAGLPYGANKDGIIWVATEGALNTPKDHIGTRNPANNAAIVLQLPQGTTLPKGFYAEGSRGGSQASSRSSSRSRNSSRNSTPGSSRGTSPARMAGNGGDAALALLLLDRLNQLESKMSGKGQQQQGQTVTKKSAAEASKKPRQKRTATKAYNVTQAFGRRGPEQTQGNFGDQELIRQGTDYKHWPQIAQFAPSASAFFGMSRIGMEVTPSGTWLTYTGAIKLDDKDPNFKDQVILLNKHIDAYKTFPPTEPKKDKKKKADETQALPQRQKKQQTVTLLPAADLDDFSKQLQQSMSSADSTQA

SEQ ID NO: 22 - protein, 174 aa, Unknown
  SARS-CoV-2
MSDNGPQNQRNAPRITFGGPSDSTGSNQNGERSGARSKQRRPQGLPNNTASWFTALTQHGKEDLKFPRGQGVPINTNSSPDDQIGYYRRATRRIRGGDGKMKDLSPRWYFYYLGTGPEAGLPYGANKDGIIWVATEGALNTPKDHIGTRNPANNAAIVLQLPQGTTLPKGFYAE

SEQ ID NO: 23 - protein, 73 aa, Unknown
  SARS-CoV-2
GSRGGSQASSRSSSRSRNSSRNSTPGSSRGTSPARMAGNGGDAALALLLLDRLNQLESKMSGKGQQQQGQTVT

SEQ ID NO: 24 - protein, 172 aa, Unknown
  SARS-CoV-2
KKSAAEASKKPRQKRTATKAYNVTQAFGRRGPEQTQGNFGDQELIRQGTDYKHWPQIAQFAPSASAFFGMSRIGMEVTPSGTWLTYTGAIKLDDKDPNFKDQVILLNKHIDAYKTFPPTEPKKDKKKKADETQALPQRQKKQQTVTLLPAADLDDFSKQLQQSMSSADSTQA

SEQ ID NO: 25 - protein, 5 aa, Unknown
  SARS-CoV-2
LLPAA

SEQ ID NO: 26 - protein, 9 aa, Unknown
  SARS-CoV-2
LDDFSKQLQ

SEQ ID NO: 27 - protein, 9 aa, Unknown
  SARS-CoV-2
QLQQSMSSA

SEQ ID NO: 28 - protein, 21 aa, Unknown
  SARS-CoV-2
KQQTVTLLPAADLDDFSKQLQ

SEQ ID NO: 29 - protein, 9 aa, Unknown
  SARS-CoV-2
LDDFSKQLQ

SEQ ID NO: 30 - protein, 18 aa, Unknown
  SARS-CoV-2
AADLDDFSKQLQQSMSSA

SEQ ID NO: 31 - protein, 18 aa, Unknown
  peptide 1
ARMAGNGGDAALALLLLD

SEQ ID NO: 32 - protein, 19 aa, Unknown
  peptide 2
TAALALLLLDRLNQLESKM

SEQ ID NO: 33 - protein, 18 aa, Unknown
  peptide 3
RLNQLESKMSGKGQQQQG

SEQ ID NO: 34 - protein, 18 aa, Unknown
  peptide 4
SGKGQQQQGQTVTKKSAA

SEQ ID NO: 35 - protein, 18 aa, Unknown
  peptide 5
QTVTKKSAAEASKKPRQK

SEQ ID NO: 36 - protein, 18 aa, Unknown
  peptide 6
EASKKPRQKRTATKAYNV

SEQ ID NO: 37 - protein, 18 aa, Unknown
  peptide 7
RTATKAYNVTQAFGRRGP

SEQ ID NO: 38 - protein, 18 aa, Unknown
  peptide 8
TQAFGRRGPEQTQGNFGD

SEQ ID NO: 39 - protein, 18 aa, Unknown
  peptide 9
EQTQGNFGDQELIRQGTD

SEQ ID NO: 40 - protein, 18 aa, Unknown
  peptide 10
QELIRQGTDYKHWPQIAQ

SEQ ID NO: 41 - protein, 18 aa, Unknown
  peptide 11
YKHWPQIAQFAPSASAFF

SEQ ID NO: 42 - protein, 18 aa, Unknown
  peptide 12
FAPSASAFFGMSRIGMEV

SEQ ID NO: 43 - protein, 18 aa, Unknown
  peptide 13
GMSRIGMEVTPSGTWLTY

SEQ ID NO: 44 - protein, 18 aa, Unknown
  peptide 14
TPSGTWLTYTGAIKLDDK

SEQ ID NO: 45 - protein, 18 aa, Unknown
  peptide 15
TGAIKLDDKDPNFKDQVI

SEQ ID NO: 46 - protein, 18 aa, Unknown
  peptide 16
DPNFKDQVILLNKHIDAY

SEQ ID NO: 47 - protein, 19 aa, Unknown
  peptide 17
LLNKHIDAYKITFPPTEPK

SEQ ID NO: 48 - protein, 18 aa, Unknown
  peptide 18
KTFPPTEPKKDKKKKADE

SEQ ID NO: 49 - protein, 18 aa, Unknown
  peptide 19
KDKKKKADETQALPQRQK

SEQ ID NO: 50 - protein, 18 aa, Unknown
  peptide 20
TQALPQRQKKQQTVTLLP

SEQ ID NO: 51 - protein, 18 aa, Unknown
  peptide 21
KQQTVTLLPAADLDDFSK

SEQ ID NO: 52 - protein, 18 aa, Unknown
  peptide 22
AADLDDFSKQLQQSMSSA

SEQ ID NO: 53 - protein, 14 aa, Unknown
  peptide 23
QLQQSMSSADSTQA

SEQ ID NO: 54 - protein, 7 aa, Unknown
  peptide 24
RQKKQQT

SEQ ID NO: 55 - protein, 7 aa, Unknown
  peptide 25
QKKQQTV

SEQ ID NO: 56 - protein, 7 aa, Unknown
  peptide 26
KKQQTVT

SEQ ID NO: 57 - protein, 7 aa, Unknown
  peptide 27
KQQTVTL

SEQ ID NO: 58 - protein, 7 aa, Unknown
  peptide 28
QQTVTLL

SEQ ID NO: 59 - protein, 7 aa, Unknown
  peptide 29
QTVTLLP

SEQ ID NO: 60 - protein, 7 aa, Unknown
  peptide 30
TVTLLPA

SEQ ID NO: 61 - protein, 7 aa, Unknown
  peptide 31
VTLLPAA

SEQ ID NO: 62 - protein, 7 aa, Unknown
  peptide 32
TLLPAAD

SEQ ID NO: 63 - protein, 7 aa, Unknown
  peptide 33
LLPAADL

SEQ ID NO: 64 - protein, 7 aa, Unknown
  peptide 34
LPAADLD

SEQ ID NO: 65 - protein, 7 aa, Unknown
  peptide 35
PAADLDD

SEQ ID NO: 66 - protein, 7 aa, Unknown
  peptide 36
AADIDDF

SEQ ID NO: 67 - protein, 7 aa, Unknown
  peptide 37
ADLDDFS

SEQ ID NO: 68 - protein, 7 aa, Unknown
  peptide 38
DLDDESK

SEQ ID NO: 69 - protein, 7 aa, Unknown
  peptide 39
LDDFSKQ

SEQ ID NO: 70 - protein, 15 aa, Unknown
  peptide 40
QQTVTLLPAADLDDF

SEQ ID NO: 71 - protein, 15 aa, Unknown
  ptide 41
QTVTLLPAADLDDFS

SEQ ID NO: 72 - protein, 15 aa, Unknown
  eptide 42
TVTLLPAADLDDFSK

SEQ ID NO: 73 - protein, 15 aa, Unknown
  peptide 43
VTLLPAADLDDESKQ

SEQ ID NO: 74 - protein, 15 aa, Unknown
  peptide 44
TLLPAADLDDFSKQL

SEQ ID NO: 75 - protein, 15 aa, Unknown
  peptide 45
LLPAADLDDESKQLQ

SEQ ID NO: 76 - protein, 15 aa, Unknown
  peptide 46
LPAADLDDFSKQLQQ

SEQ ID NO: 77 - protein, 15 aa, Unknown
  peptide 47
PAADLDDFSKQLQQS

SEQ ID NO: 78 - protein, 15 aa, Unknown
  peptide 48
PAADLDDFSKQLQQS

SEQ ID NO: 79 - protein, 15 aa, Unknown
  peptide 49
ADLDDFSKQLQQSMS

SEQ ID NO: 80 - protein, 15 aa, Unknown
  peptide 50
DLDDFSKQLQQSMSS

SEQ ID NO: 81 - protein, 15 aa, Unknown
  peptide 51
LDDFSKQLQQSMSSA

SEQ ID NO: 82 - protein, 15 aa, Unknown
  peptide 52
DDFSKQLQQSMSSAD

SEQ ID NO: 83 - protein, 15 aa, Unknown
  peptide 53
DFSKQLQQSMSSADS

SEQ ID NO: 84 - protein, 15 aa, Unknown
  peptide 54
FSKQLQQSMSSADST

SEQ ID NO: 85 - protein, 15 aa, Unknown
  peptide 55
SKQLQQSMSSADSTQ